European Patent Specification EP 4 100 532 B1, published August 12, 2026. Title: AAV-NAGLU Vectors for Treatment of Mucopolysaccharidosis IIIB. Applicant: The University of North Carolina at Chapel Hill Fu, Haiyan Bobo, Tierra. The sequence listing filed with the application follows.

SEQUENCE LISTING (4 sequences)

SEQ ID NO: 1 - DNA, 2232 bp, Artificial
  codon-optimized alpha-N-acetylglucosaminidase
atggaggctgttgctgttgcagccgctgtgggcgtcttgctgttggccggtgccgggggagctgctggcgacgaggcaagggaagctgcagctgtgcgggctctcgtcgcaaggttgctgggtccaggtcccgctgctgactttagtgtgtcagtggagagggctttggccgctaaacctggcctggacacctactccctgggtggaggtggggctgcccgcgtgagggtgagaggctcaacgggggtggctgctgcagcaggtctgcataggtacctcagagacttctgcggatgccatgtcgcttggagcggcagtcaactgaggctgccccggcccctccctgccgtccctggggaacttacagaagctactccaaataggtacagatattatcaaaatgtgtgtacgcagagttacagctttgtgtggtgggactgggcaaggtgggagcgcgaaatcgattggatggccctcaacgggatcaatctggccttggcatggtccggacaggaagctatctggcagcgcgtgtatctggctctcgggttgactcaagctgaaatcaacgagtttttcacaggccccgccttcctggcctgggggcggatgggtaatcttcatacttgggacgggccactgcccccctcttggcacatcaaacagttgtatctgcagcaccgcgtcctggaccagatgcgcagcttcggcatgactcccgtcctgccggctttcgcagggcacgtcccagaggcggtcacacgggtcttccctcaggtgaatgtgacaaaaatgggatcatggggacatttcaattgttcttacagttgttccttcctgctggcacccgaagatcctatcttcccaatcataggaagtctctttctgcgcgagttgattaaggagttcggtactgatcacatttatggcgctgatacttttaacgaaatgcagcccccctcttctgaaccatcctatcttgctgccgcaaccactgccgtttatgaagccatgaccgccgtggacactgaagccgtttggcttctccaaggttggctgttccagcaccagcctcagttttgggggccagctcagataagagccgttctcggcgctgtacctcgcggaagactgctggtgcttgatttgttcgcagagtctcagccagtgtacacgagaaccgcttccttccagggccagccgtttatttggtgtatgcttcacaattttggcggaaatcatgggctgttcggtgccctggaggccgtcaatgggggacctgaggctgcaagattgttcccaaactcaaccatggtggggaccggaatggcacccgaaggcattagccagaatgaggtcgtctacagtctgatggcggaattggggtggcggaaggaccccgtgccagatctcgccgcctgggtgactagctttgccgcccgccgctatggagtgagccatcctgatgcaggcgcagcctggcggctgttgcttcgatcagtatacaattgttcaggagaggcctgccgggggcacaataggagcccactggtaaggaggcccagcctgcagatgaacacctctatctggtacaacagaagcgatgttttcgaggcttggagacttctccttacatctgcccctagcttggccaccagtccagccttccgatatgatctgctggacctcacccgacaggccgtgcaggaactggtctctctctactatgaagaggccagatcagcttacctctctaaagaactggcctccctcttgcgagcaggaggcgtcctggcatatgagctgctccctgcactggacgaggtactggcatctgattcccgattcctgctcgggtcatggctggagcaagcccgagcagcggctgtaagcgaggctgaagcagacttctatgaacaaaatagtaggtatcaactgactctgtggggtccagaggggaatatcctggactacgcgaacaaacagttggcgggcctggtggccaactactacacccctcggtggagattgtttttggaggcgctggtggattcagtcgcacaggggattccgtttcagcaacatcagtttgacaagaacgtctttcagctggaacaggcttttgtgctttctaagcagcgctacccttctcagccaagaggcgataccgttgacctcgcgaagaaaatctttctcaagtactatcccagatgggtggccggatcatggtag

SEQ ID NO: 2 - DNA, 2232 bp, Homo sapiens
atggaggcggtggcggtggccgcggcggtgggggtccttctcctggccggggccgggggcgcggcaggcgacgaggcccgggaggcggcggccgtgcgggcgctcgtggcccggctgctggggccaggccccgcggccgacttctccgtgtcggtggagcgcgctctggctgccaagccgggcttggacacctacagcctgggcggcggcggcgcggcgcgcgtgcgggtgcgcggctccacgggcgtggcggccgccgcggggctgcaccgctacctgcgcgacttctgtggctgccacgtggcctggtccggctctcagctgcgcctgccgcggccactgccagccgtgccgggggagctgaccgaggccacgcccaacaggtaccgctattaccagaatgtgtgcacgcaaagctactccttcgtgtggtgggactgggcccgctgggagcgagagatagactggatggcgctgaatggcatcaacctggcactggcctggagcggccaggaggccatctggcagcgggtgtacctggccttgggcctgacccaggcagagatcaatgagttctttactggtcctgccttcctggcctgggggcgaatgggcaacctgcacacctgggatggccccctgcccccctcctggcacatcaagcagctttacctgcagcaccgggtcctggaccagatgcgctccttcggcatgaccccagtgctgcctgcattcgcggggcatgttcccgaggctgtcaccagggtgttccctcaggtcaatgtcacgaagatgggcagttggggccactttaactgttcctactcctgctccttccttctggctccggaagaccccatattccccatcatcgggagcctcttcctgcgagagctgatcaaagagtttggcacagaccacatctatggggccgacactttcaatgagatgcagccaccttcctcagagccctcctaccttgccgcagccaccactgccgtctatgaggccatgactgcagtggatactgaggctgtgtggctgctccaaggctggctcttccagcaccagccgcagttctgggggcccgcccagatcagggctgtgctgggagctgtgccccgtggccgcctcctggttctggacctgtttgctgagagccagcctgtgtatacccgcactgcctccttccagggccagcccttcatctggtgcatgctgcacaactttgggggaaaccatggtctttttggagccctagaggctgtgaacggaggcccagaagctgcccgcctcttccccaactccaccatggtaggcacgggcatggcccccgagggcatcagccagaacgaagtggtctattccctcatggctgagctgggctggcgaaaggacccagtgccagatttggcagcctgggtgaccagctttgccgcccggcggtatggggtctcccacccggacgcaggggcagcgtggaggctactgctccggagtgtgtacaactgctccggggaggcctgcaggggccacaatcgtagcccgctggtcaggcggccgtccctacagatgaataccagcatctggtacaaccgatctgatgtgtttgaggcctggcggctgctgctcacatctgctccctccctggccaccagccccgccttccgctacgacctgctggacctcactcggcaggcagtgcaggagctggtcagcttgtactatgaggaggcaagaagcgcctacctgagcaaggagctggcctccctgttgagggctggaggcgtcctggcctatgagctgctgccggcactggacgaggtgctggctagtgacagccgcttcttgctgggcagctggctagagcaggcccgagcagcggcagtcagtgaggccgaggccgatttctacgagcagaacagccgctaccagctgaccttgtgggggccagaaggcaacatcctggactatgccaacaagcagctggcggggttggtggccaactactacacccctcgctggcggcttttcctggaggcgctggttgacagtgtggcccagggcatccctttccaacagcaccagtttgacaaaaatgtcttccaactggagcaggccttcgttctcagcaagcagaggtaccccagccagccgcgaggagacactgtggacctggccaagaagatcttcctcaaatattaccccggctgggtggccggctcttggtga

SEQ ID NO: 3 - DNA, 7730 bp, Artificial
  plasmid
ggggggggggggggggggttggccactccctctctgcgcgctcgctcgctcactgaggccgggcgaccaaaggtcgcccgacgcccgggctttgcccgggcggcctcagtgagcgagcgagcgcgcagagagggagtggccaactccatcactaggggttcctagatctggaagctgatcttcaatattggccattagccatattattcattggttatatagcataaatcaatattggatattggccattgcatacgttgtatctatatcataatatgtacatttatattggctcatgtccaatatgaccgccatgttggcattgattattgactagttattaatagtaatcaattacggggtcattagttcatagcccatatatggagttccgcgttacataacttacggtaaatggcccgcctggctgaccgcccaacgacccccgcccattgacgtcaataatgacgtatgttcccatagtaacgccaatagggactttccattgacgtcaatgggtggagtatttacggtaaactgcccacttggcagtacatcaagtgtatcatatgccaagtccgccccctattgacgtcaatgacggtaaatggcccgcctggcattatgcccagtacatgaccttacgggactttcctacttggcagtacatctacgtattagtcatcgctattaccatggtcgaggtgagccccacgttctgcttcactctccccatctcccccccctccccacccccaattttgtatttatttattttttaattattttgtgcagcgatgggggcggggggggggggggggcgcgcgccaggcggggcggggcggggcgaggggcggggcggggcgaggcggagaggtgcggcggcagccaatcagagcggcgcgctccgaaagtttccttttatggcgaggcggcggcggcggcggccctataaaaagcgaagcgcgcggcgggcgggagtcgctgcgacgctgccttcgccccgtgccccgctccgccgccgcctcgcgccgcccgccccggctctgactgaccgcgttactcccacaggtgagcgggcgggacggcccttctcctccgggctgtaattagcgcttggtttaatgacggcttgtttcttttctgtggctgcgtgaaagccttgaggggctccgggagggccctttgtgcgggggggagcggctcggggggtgcgtgcgtgtgtgtgtgcgtggggagcgccgcgtgcggcccgcgctgcccggcggctgtgagcgctgcgggcgcggcgcggggctttgtgcgctccgcagtgtgcgcgaggggagcgcggccgggggcggtgccccgcggtgcggggggggctgcgaggggaacaaaggctgcgtgcggggtgtgtgcgtgggggggtgagcagggggtatgggcgcggcggtcgggctgtaacccccccctgcacccccctccccgagttgctgagcacggcccggcttcgggtgcggggctccgtacggggcgtggcgcggggctcgccgtgccgggcggggggtggcggcaggtgggggtgccgggcggggcggggccgcctcgggccggggagggctcgggggaggggcgcggcggcccccggagcgccggcggctgtcgaggcgcggcgagccgcagccattgccttttatggtaatcgtgcgagagggcgcagggacttactttgtcccaaatctgtgcggagccgaaatctgggaggcgccgccgcaccccctctagcgggcgcggggcgaagcggtgcggcgccggcaggaaggaaatgggcggggagggccttcgtgcgtcgccgcgccgccgtccccttctccctctccagcctcggggctgtccgcggggggacggctgccttcgggggggacggggcagggcggggttcggcttctggcgtgtgaccggcggctctagagcctctgctaaccatgttcatgccttcttctttttcctacagctcctgggcaacgtgctggttattgtgctgtctcatcattttggcaaagaattcgataggatccggtactcgaggaactgaaaaaccagaaagttaactggtaagtttagtctttttgtcttttatttcaggtcccggatccggtggtggtgcaaatcaaagaactgctcctcagtggatgttgcctttacttctaggcctgtacggaagtgttacttctgctctaaaagctgcggaattgtacccgcggcccgggatccaccggccaccggtattcgcagaccatggaggctgttgctgttgcagccgctgtgggcgtcttgctgttggccggtgccgggggagctgctggcgacgaggcaagggaagctgcagctgtgcgggctctcgtcgcaaggttgctgggtccaggtcccgctgctgactttagtgtgtcagtggagagggctttggccgctaaacctggcctggacacctactccctgggtggaggtggggctgcccgcgtgagggtgagaggctcaacgggggtggctgctgcagcaggtctgcataggtacctcagagacttctgcggatgccatgtcgcttggagcggcagtcaactgaggctgccccggcccctccctgccgtccctggggaacttacagaagctactccaaataggtacagatattatcaaaatgtgtgtacgcagagttacagctttgtgtggtgggactgggcaaggtgggagcgcgaaatcgattggatggccctcaacgggatcaatctggccttggcatggtccggacaggaagctatctggcagcgcgtgtatctggctctcgggttgactcaagctgaaatcaacgagtttttcacaggccccgccttcctggcctgggggcggatgggtaatcttcatacttgggacgggccactgcccccctcttggcacatcaaacagttgtatctgcagcaccgcgtcctggaccagatgcgcagcttcggcatgactcccgtcctgccggctttcgcagggcacgtcccagaggcggtcacacgggtcttccctcaggtgaatgtgacaaaaatgggatcatggggacatttcaattgttcttacagttgttccttcctgctggcacccgaagatcctatcttcccaatcataggaagtctctttctgcgcgagttgattaaggagttcggtactgatcacatttatggcgctgatacttttaacgaaatgcagcccccctcttctgaaccatcctatcttgctgccgcaaccactgccgtttatgaagccatgaccgccgtggacactgaagccgtttggcttctccaaggttggctgttccagcaccagcctcagttttgggggccagctcagataagagccgttctcggcgctgtacctcgcggaagactgctggtgcttgatttgttcgcagagtctcagccagtgtacacgagaaccgcttccttccagggccagccgtttatttggtgtatgcttcacaattttggcggaaatcatgggctgttcggtgccctggaggccgtcaatgggggacctgaggctgcaagattgttcccaaactcaaccatggtggggaccggaatggcacccgaaggcattagccagaatgaggtcgtctacagtctgatggcggaattggggtggcggaaggaccccgtgccagatctcgccgcctgggtgactagctttgccgcccgccgctatggagtgagccatcctgatgcaggcgcagcctggcggctgttgcttcgatcagtatacaattgttcaggagaggcctgccgggggcacaataggagcccactggtaaggaggcccagcctgcagatgaacacctctatctggtacaacagaagcgatgttttcgaggcttggagacttctccttacatctgcccctagcttggccaccagtccagccttccgatatgatctgctggacctcacccgacaggccgtgcaggaactggtctctctctactatgaagaggccagatcagcttacctctctaaagaactggcctccctcttgcgagcaggaggcgtcctggcatatgagctgctccctgcactggacgaggtactggcatctgattcccgattcctgctcgggtcatggctggagcaagcccgagcagcggctgtaagcgaggctgaagcagacttctatgaacaaaatagtaggtatcaactgactctgtggggtccagaggggaatatcctggactacgcgaacaaacagttggcgggcctggtggccaactactacacccctcggtggagattgtttttggaggcgctggtggattcagtcgcacaggggattccgtttcagcaacatcagtttgacaagaacgtctttcagctggaacaggcttttgtgctttctaagcagcgctacccttctcagccaagaggcgataccgttgacctcgcgaagaaaatctttctcaagtactatcccagatgggtggccggatcatggtaggtcgaccctcgactagagctcgctgatcagcctcgactgtgccttctagttgccagccatctgttgtttgcccctcccccgtgccttccttgaccctggaaggtgccactcccactgtcctttcctaataaaatgaggaaattgcatcgcattgtctgagtaggtgtcattctattctggggggtggggtggggcaggacagcaagggggaggattgggaagacaatagcaggcatgctggggagagatctaggaacccctagtgatggagttggccactccctctctgcgcgctcgctcgctcactgaggccgcccgggcaaagcccgggcgtcgggcgacctttggtcgcccggcctcagtgagcgagcgagcgcgcagagagggagtggccaacccccccccccccccccctgcagccagctggcgtaatagcgaagaggcccgcaccgatcgcccttcccaacagttgcgtagcctgaatggcgaatggcgcgacgcgccctgtagcggcgcattaagcgcggcgggtgtggtggttacgcgcagcgtgaccgctacacttgccagcgccctagcgcccgctcctttcgctttcttcccttcctttctcgccacgttcgccggctttccccgtcaagctctaaatcgggggctccctttagggttccgatttagtgctttacggcacctcgaccccaaaaaacttgattagggtgatggttcacgtagtgggccatcgccctgatagacggtttttcgccctttgacgttggagtccacgttctttaatagtggactcttgttccaaactggaacaacactcaaccctatctcggtctattcttttgatttataagggattttgccgatttcggcctattggttaaaaaatgagctgatttaacaaaaatttaacgcgaattttaacaaaatattaacgtttacaatttcctgatgcggtattttctccttacgcatctgtgcggtatttcacaccgcatatggtgcactctcagtacaatctgctctgatgccgcatagttaagccagccccgacacccgccaacacccgctgacgcgccctgacgggcttgtctgctcccggcatccgcttacagacaagctgtgaccgtctccgggagctgcatgtgtcagaggttttcaccgtcatcaccgaaacgcgcgagacgaaagggcctcgtgatacgcctatttttataggttaatgtcatgataataatggtttcttagacgtcaggtggcacttttcggggaaatgtgcgcggaacccctatttgtttatttttctaaatacattcaaatatgtatccgctcatgagacaataaccctgataaatgcttcaataatattgaaaaaggaagagtatgagtattcaacatttccgtgtcgcccttattcccttttttgcggcattttgccttcctgtttttgctcacccagaaacgctggtgaaagtaaaagatgctgaagatcagttgggtgcacgagtgggttacatcgaactggatctcaacagcggtaagatccttgagagttttcgccccgaagaacgttttccaatgatgagcacttttaaagttctgctatgtggcgcggtattatcccgtattgacgccgggcaagagcaactcggtcgccgcatacactattctcagaatgacttggttgagtactcaccagtcacagaaaagcatcttacggatggcatgacagtaagagaattatgcagtgctgccataaccatgagtgataacactgcggccaacttacttctgacaacgatcggaggaccgaaggagctaaccgcttttttgcacaacatgggggatcatgtaactcgccttgatcgttgggaaccggagctgaatgaagccataccaaacgacgagcgtgacaccacgatgcctgtagcaatggcaacaacgttgcgcaaactattaactggcgaactacttactctagcttcccggcaacaattaatagactggatggaggcggataaagttgcaggaccacttctgcgctcggcccttccggctggctggtttattgctgataaatctggagccggtgagcgtgggtctcgcggtatcattgcagcactggggccagatggtaagccctcccgtatcgtagttatctacacgacggggagtcaggcaactatgaccttccagggtcaaggaagctgtcagaccaagtttactcatatatactttagattgatttaaaacttcatttttaatttaaaaggatctaggtgaagatcctttttgataatctcatgaccaaaatcccttaacgtgagttttcgttccactgagcgtcagaccccgtagaaaagatcaaaggatcttcttgagatcctttttttctgcgcgtaatctgctgcttgcaaacaaaaaaaccaccgctaccagcggtggtttgtttgccggatcaagagctaccaactctttttccgaaggtaactggcttcagcagagcgcagataccaaatactgtccttctagtgtagccgtagttaggccaccacttcaagaactctgtagcaccgcctacatacctcgctctgctaatcctgttaccagtggctgctgccagtggcgataagtcgtgtcttaccgggttggactcaagacgatagttaccggataaggcgcagcggtcgggctgaacggggggttcgtgcacacagcccagcttggagcgaacgacctacaccgaactgagatacctacagcgtgagcattgagaaagcgccacgcttcccgaagggagaaaggcggacaggtatccggtaagcggcagggtcggaacaggagagcgcacgagggagcttccagggggaaacgcctggtatctttatagtcctgtcgggtttcgccacctctgacttgagcgtcgatttttgtgatgctcgtcaggggggcggagcctatggaaaaacgccagcaacgcggcctttttacggttcctggccttttgctggccttttgctcacatgttctttcctgcgttatcccctgattctgtggataaccgtattaccgcctttgagtgagctgataccgctcgccgcagccgaacgaccgagcgcagcgagtcagtgagcgaggaagcggaagagcgcccaatacgcaaaccgcctctccccgcgcgttggccgattcattaatgcagctgggctgca

SEQ ID NO: 4 - DNA, 6460 bp, Artificial
  plasmid
ggggggggggggggggggttggccactccctctctgcgcgctcgctcgctcactgaggccgggcgaccaaaggtcgcccgacgcccgggctttgcccgggcggcctcagtgagcgagcgagcgcgcagagagggagtggccaactccatcactaggggttcctagatctgaattcggtacccgttacataacttacggtaaatggcccgcctggctgaccgcccaacgacccccgcccattgacgtcaataatgacgtatgttcccatagtaacgccaatagggactttccattgacgtcaatgggtggagtatttacggtaaactgcccacttggcagtacatcaagtgtatcatatgccaagtacgccccctattgacgtcaatgacggtaaatggcccgcctggcattatgcccagtacatgaccttatgggactttcctacttggcagtacatctacgtattagtcatcgctattaccatggtgatgcggttttggcagtacatcaatgggcgtggatagcggtttgactcacggggatttccaagtctccaccccattgacgtcaatgggagtttgttttggcaccaaaatcaacgggactttccaaaatgtcgtaacaactccgccccattgacgcaaatgggcggtaggcgtgtacggtgggaggtctatataagcagagctcgtttagtgaaccgtcagatcgcctggagacgccatccacgctgttttgacctccatagaagacaccgggaccgatccagcctccggactctagaggatccggtactcgaggaactgaaaaaccagaaagttaactggtaagtttagtctttttgtcttttatttcaggtcccggatccggtggtggtgcaaatcaaagaactgctcctcagtggatgttgcctttacttctaggcctgtacggaagtgttacttctgctctaaaagctgcggaattgtacccgcggcccgggatccaccggccaccggtattcgcagaccatggaggctgttgctgttgcagccgctgtgggcgtcttgctgttggccggtgccgggggagctgctggcgacgaggcaagggaagctgcagctgtgcgggctctcgtcgcaaggttgctgggtccaggtcccgctgctgactttagtgtgtcagtggagagggctttggccgctaaacctggcctggacacctactccctgggtggaggtggggctgcccgcgtgagggtgagaggctcaacgggggtggctgctgcagcaggtctgcataggtacctcagagacttctgcggatgccatgtcgcttggagcggcagtcaactgaggctgccccggcccctccctgccgtccctggggaacttacagaagctactccaaataggtacagatattatcaaaatgtgtgtacgcagagttacagctttgtgtggtgggactgggcaaggtgggagcgcgaaatcgattggatggccctcaacgggatcaatctggccttggcatggtccggacaggaagctatctggcagcgcgtgtatctggctctcgggttgactcaagctgaaatcaacgagtttttcacaggccccgccttcctggcctgggggcggatgggtaatcttcatacttgggacgggccactgcccccctcttggcacatcaaacagttgtatctgcagcaccgcgtcctggaccagatgcgcagcttcggcatgactcccgtcctgccggctttcgcagggcacgtcccagaggcggtcacacgggtcttccctcaggtgaatgtgacaaaaatgggatcatggggacatttcaattgttcttacagttgttccttcctgctggcacccgaagatcctatcttcccaatcataggaagtctctttctgcgcgagttgattaaggagttcggtactgatcacatttatggcgctgatacttttaacgaaatgcagcccccctcttctgaaccatcctatcttgctgccgcaaccactgccgtttatgaagccatgaccgccgtggacactgaagccgtttggcttctccaaggttggctgttccagcaccagcctcagttttgggggccagctcagataagagccgttctcggcgctgtacctcgcggaagactgctggtgcttgatttgttcgcagagtctcagccagtgtacacgagaaccgcttccttccagggccagccgtttatttggtgtatgcttcacaattttggcggaaatcatgggctgttcggtgccctggaggccgtcaatgggggacctgaggctgcaagattgttcccaaactcaaccatggtggggaccggaatggcacccgaaggcattagccagaatgaggtcgtctacagtctgatggcggaattggggtggcggaaggaccccgtgccagatctcgccgcctgggtgactagctttgccgcccgccgctatggagtgagccatcctgatgcaggcgcagcctggcggctgttgcttcgatcagtatacaattgttcaggagaggcctgccgggggcacaataggagcccactggtaaggaggcccagcctgcagatgaacacctctatctggtacaacagaagcgatgttttcgaggcttggagacttctccttacatctgcccctagcttggccaccagtccagccttccgatatgatctgctggacctcacccgacaggccgtgcaggaactggtctctctctactatgaagaggccagatcagcttacctctctaaagaactggcctccctcttgcgagcaggaggcgtcctggcatatgagctgctccctgcactggacgaggtactggcatctgattcccgattcctgctcgggtcatggctggagcaagcccgagcagcggctgtaagcgaggctgaagcagacttctatgaacaaaatagtaggtatcaactgactctgtggggtccagaggggaatatcctggactacgcgaacaaacagttggcgggcctggtggccaactactacacccctcggtggagattgtttttggaggcgctggtggattcagtcgcacaggggattccgtttcagcaacatcagtttgacaagaacgtctttcagctggaacaggcttttgtgctttctaagcagcgctacccttctcagccaagaggcgataccgttgacctcgcgaagaaaatctttctcaagtactatcccagatgggtggccggatcatggtaggtcgaccctcgactagagctcgctgatcagcctcgactgtgccttctagttgccagccatctgttgtttgcccctcccccgtgccttccttgaccctggaaggtgccactcccactgtcctttcctaataaaatgaggaaattgcatcgcattgtctgagtaggtgtcattctattctggggggtggggtggggcaggacagcaagggggaggattgggaagacaatagcaggcatgctggggagagatctaggaacccctagtgatggagttggccactccctctctgcgcgctcgctcgctcactgaggccgcccgggcaaagcccgggcgtcgggcgacctttggtcgcccggcctcagtgagcgagcgagcgcgcagagagggagtggccaacccccccccccccccccctgcagccagctggcgtaatagcgaagaggcccgcaccgatcgcccttcccaacagttgcgtagcctgaatggcgaatggcgcgacgcgccctgtagcggcgcattaagcgcggcgggtgtggtggttacgcgcagcgtgaccgctacacttgccagcgccctagcgcccgctcctttcgctttcttcccttcctttctcgccacgttcgccggctttccccgtcaagctctaaatcgggggctccctttagggttccgatttagtgctttacggcacctcgaccccaaaaaacttgattagggtgatggttcacgtagtgggccatcgccctgatagacggtttttcgccctttgacgttggagtccacgttctttaatagtggactcttgttccaaactggaacaacactcaaccctatctcggtctattcttttgatttataagggattttgccgatttcggcctattggttaaaaaatgagctgatttaacaaaaatttaacgcgaattttaacaaaatattaacgtttacaatttcctgatgcggtattttctccttacgcatctgtgcggtatttcacaccgcatatggtgcactctcagtacaatctgctctgatgccgcatagttaagccagccccgacacccgccaacacccgctgacgcgccctgacgggcttgtctgctcccggcatccgcttacagacaagctgtgaccgtctccgggagctgcatgtgtcagaggttttcaccgtcatcaccgaaacgcgcgagacgaaagggcctcgtgatacgcctatttttataggttaatgtcatgataataatggtttcttagacgtcaggtggcacttttcggggaaatgtgcgcggaacccctatttgtttatttttctaaatacattcaaatatgtatccgctcatgagacaataaccctgataaatgcttcaataatattgaaaaaggaagagtatgagtattcaacatttccgtgtcgcccttattcccttttttgcggcattttgccttcctgtttttgctcacccagaaacgctggtgaaagtaaaagatgctgaagatcagttgggtgcacgagtgggttacatcgaactggatctcaacagcggtaagatccttgagagttttcgccccgaagaacgttttccaatgatgagcacttttaaagttctgctatgtggcgcggtattatcccgtattgacgccgggcaagagcaactcggtcgccgcatacactattctcagaatgacttggttgagtactcaccagtcacagaaaagcatcttacggatggcatgacagtaagagaattatgcagtgctgccataaccatgagtgataacactgcggccaacttacttctgacaacgatcggaggaccgaaggagctaaccgcttttttgcacaacatgggggatcatgtaactcgccttgatcgttgggaaccggagctgaatgaagccataccaaacgacgagcgtgacaccacgatgcctgtagcaatggcaacaacgttgcgcaaactattaactggcgaactacttactctagcttcccggcaacaattaatagactggatggaggcggataaagttgcaggaccacttctgcgctcggcccttccggctggctggtttattgctgataaatctggagccggtgagcgtgggtctcgcggtatcattgcagcactggggccagatggtaagccctcccgtatcgtagttatctacacgacggggagtcaggcaactatgaccttccagggtcaaggaagctgtcagaccaagtttactcatatatactttagattgatttaaaacttcatttttaatttaaaaggatctaggtgaagatcctttttgataatctcatgaccaaaatcccttaacgtgagttttcgttccactgagcgtcagaccccgtagaaaagatcaaaggatcttcttgagatcctttttttctgcgcgtaatctgctgcttgcaaacaaaaaaaccaccgctaccagcggtggtttgtttgccggatcaagagctaccaactctttttccgaaggtaactggcttcagcagagcgcagataccaaatactgtccttctagtgtagccgtagttaggccaccacttcaagaactctgtagcaccgcctacatacctcgctctgctaatcctgttaccagtggctgctgccagtggcgataagtcgtgtcttaccgggttggactcaagacgatagttaccggataaggcgcagcggtcgggctgaacggggggttcgtgcacacagcccagcttggagcgaacgacctacaccgaactgagatacctacagcgtgagcattgagaaagcgccacgcttcccgaagggagaaaggcggacaggtatccggtaagcggcagggtcggaacaggagagcgcacgagggagcttccagggggaaacgcctggtatctttatagtcctgtcgggtttcgccacctctgacttgagcgtcgatttttgtgatgctcgtcaggggggcggagcctatggaaaaacgccagcaacgcggcctttttacggttcctggccttttgctggccttttgctcacatgttctttcctgcgttatcccctgattctgtggataaccgtattaccgcctttgagtgagctgataccgctcgccgcagccgaacgaccgagcgcagcgagtcagtgagcgaggaagcggaagagcgcccaatacgcaaaccgcctctccccgcgcgttggccgattcattaatgcagctgggctgca